European Patent Specification EP 3 145 947 B1, published February 12, 2025. Title: RECOMBINANT MICROORGANISMS CAPABLE OF CARBON FIXATION. Applicant: Yeda Research and Development Co. Ltd. MILO, Ron ANTONOVSKY, Niv NOOR, Elad BAR-EVEN, Arren ZOHAR, Yehudit ZELCBUCH, Lior GLEIZER, Shmuel AMRAM, Shira. The sequence listing filed with the application follows.

SEQUENCE LISTING (27 sequences)

SEQ ID NO: 1 - DNA, 1422 bp, Rhodospirillum rubrum
atgcatcatcaccatcaccacatggaccagtcatctcgttacgtcaatctggcgctcaaggaagaggatctgatcgccggcggcgagcatgtgctttgtgcctatatcatgaagcccaaggccggatatggctatgtggcgaccgcggcgcatttcgccgccgagagttcgacgggcaccaacgtcgaggtctgcaccaccgacgatttcacccggggcgtcgacgccctggtctatgaggtggacgaggcccgcgagctgaccaagatcgcctatccggtggctttgttcgaccgcaacatcaccgacggcaaggcgatgatcgcctcgttcctgacgctcaccatgggaaacaaccagggtatgggcgacgtggaatacgccaagatgcacgatttctatgtgcccgaggcttatcgcgccctgtttgatggcccgagcgtcaatatctcggccctgtggaaagtgctggggcggcccgaggtcgacggcggtctggtcgtcggcacgatcatcaagccgaagctcggcctgcgtcccaagcccttcgccgaggcctgccacgccttctggctgggcggcgacttcatcaagaacgacgagccccagggcaatcagcccttcgcccccttgcgcgacaccatcgccctggtcgccgacgccatgaggcgggcccaggacgagaccggcgaggccaagctgttctcggccaatatcaccgccgacgatcccttcgagatcatcgcccgtggcgagtatgtgctggagaccttcggcgagaacgcctcgcatgtcgccttgctggtcgacggctatgtcgccggcgccgcggcgatcaccacggcgcgccgccgcttccccgataacttcttgcattatcaccgggctggccacggcgccgtcacctcgccccagtccaagcgcggctataccgccttcgtccattgcaagatggcccgccttcaaggcgccagcggcatccacaccggcaccatgggctttggcaagatggaaggcgagtccagcgaccgcgccatcgcctatatgctgacccaggacgaggcccaggggccgttctaccgtcaatcctggggcggcatgaaggcttgtacgccgatcatcagcggcggcatgaacgccctgcgcatgcccggcttcttcgagaacctgggtaatgccaatgtcatcttgaccgccggcggcggcgccttcggccatatcgacggcccggtggccggggcgcggtcgttgcgtcaagcctggcaagcctggcgggacggggttccggttctggactatgcccgcgagcacaaggaactggcccgcgccttcgagtccttccccggcgacgccgaccagatctatccgggctggcgcaaggccctgggcgtcgaggacacccgcagcgcccttccggcgtaa

SEQ ID NO: 2 - DNA, 1019 bp, Synechococcus elongatus
tgcatcatcaccatcaccacagcaagccagatcgtgttgttttgatcggcgttgccggtgactccggttgcggcaaatcaaccttcctaaatcgccttgccgacttgtttggtacggaattgatgacggtcatctgcttggatgactatcacagtctcgatcgcaagggccggaaggaagcaggcgtaacggctttggatccccgcgccaacaactttgacttgatgtatgaacaggtcaaggcgttgaagaacggcgaaacgatcatgaagccgatctacaaccatgaaaccggcttgatcgatccgcccgaaaaaatcgaacccaatcgcatcattgtgatcgagggtctgcatccgctttacgacgagcgcgtgcgtgaactgctcgatttcagcgtttacctcgacatcgatgacgaagtcaaaatcgcttggaagatccaacgcgatatggcagaacgcggccactcctacgaagatgtcctcgcctcgatcgaagcgcgccgccctgacttcaaggcctacattgagccccagcgtggccatgcggacatcgtcatccgcgtcatgccgacccagctaatccccaatgacaccgagcgcaaggtgctgcgggtgcagttgatccaacgggaaggccgcgatggttttgagccggcttacctgttcgacgaaggttcgaccatccagtggacgccctgcggtcgtaagctgacctgctcctatccgggcattcgcttagcctacggccctgacacctactacggtcacgaagtctcagtgcttgaggtcgacggtcagttcgagaacctcgaagagatgatctacgtcgagggccacctcagcaagaccgacacgcagtactacggtgagttgacccacctgctgctacagcacaaagattacccgggttcgaacaacggcacgggtctgttccaagtgctgaccggcctgaaaatgcgggcggcctatgagcgtttgacctcccaagcagcacccgtcgccgctagtgtctag

SEQ ID NO: 3 - DNA, 660 bp, Rhodospirillum rubrum
atgcatcatcaccatcaccacgacatccaggatctcattaccaacaatcggaaatgggccgaggagcgcgaatccgcccttcctggctattttcatatcctcagcgaagtgcagtcgccgaagtttttgtggatcggctgctcggactcgcgggtgccggccaatgaaatcgtcggcatgcagccgggcgaacttttcgttcaccgcaacatcgccaacgttgttccccatgccgacgccaattgccacgccgtgctcgaatacgccatcgacgtgctgaaggtcgagcacatcatggtcgtcggccattacggctgcggcggggttcgcgccgccctgaaccgtctggccatggggccgatcgacaactggctgtcccacatcaaggacatcgcccgtatcttcgccgccgagctggaagacctacccgacgaggaaagccgggtcgaccggctgtgcgaactcaacgccatggcccaggtgatgaacgtggcgcgcacctcgatggttcaggcggcttggcgacgcggccagcctttggccatccacgcttggtgctatggtctgaagactgggctggtcaatgatcttggccgaaccctaacccgcatcgccgatctgcccgaaccctatcggctgatctttcccgatcaggtctaa

SEQ ID NO: 4 - protein, 466 aa, Rhodospirillum rubrum
MDQSSRYVNLALKEEDLIAGGEHVLCAYIMKPKAGYGYVATAAHFAAESSTGTNVEVCTTDDFTRGVDALVYEVDEARELTKIAYPVALFDRNITDGKAMIASFLTLTMGNNQGMGDVEYAKMHDFYVPEAYRALFDGPSVNISALWKVLGRPEVDGGLVVGTIIKPKLGLRPKPFAEACHAFWLGGDFIKNDEPQGNQPFAPLRDTIALVADAMRRAQDETGEAKLFSANITADDPFEIIARGEYVLETFGENASHVALLVDGYVAGAAAITTARRRFPDNFLHYHRAGHGAVTSPQSKRGYTAFVHCKMARLQGASGIHTGTMGFGKMEGESSDRAIAYMLTQDEAQGPFYRQSWGGMKACTPIISGGMNALRMPGFFENLGNANVILTAGGGAFGHIDGPVAGARSLRQAWQAWRDGVPVLDYAREHKELARAFESFPGDADQIYPGWRKALGVEDTRSALPA

SEQ ID NO: 5 - protein, 333 aa, Synechococcus elongatus
MSKPDRVVLIGVAGDSGCGKSTFLNRLADLFGTELMTVICLDDYHSLDRKGRKEAGVTALDPRANNFDLMYEQVKALKNGETIMKPIYNHETGLIDPPEKIEPNRIIVIEGLHPLYDERVRELLDFSVYLDIDDEVKIAWKIQRDMAERGHSYEDVLASIEARRPDFKAYIEPQRGHADIVIRVMPTQLIPNDTERKVLRVQLIQREGRDGFEPAYLFDEGSTIQWTPCGRKLTCSYPGIRLAYGPDTYYGHEVSVLEVDGQFENLEEMIYVEGHLSKTDTQYYGELTHLLLQHKDYPGSNNGTGLFQVLTGLKMRAAYERLTSQAAPVAASV

SEQ ID NO: 6 - protein, 213 aa, Rhodospirillum rubrum
MDIQDLITNNRKWAEERESALPGYFHILSEVQSPKFLWIGCSDSRVPANEIVGMQPGELFVHRNIANVVPHADANCHAVLEYAIDVLKVEHIMVVGHYGCGGVRAALNRLAMGPIDNWLSHIKDIARIFAAELEDLPDEESRVDRLCELNAMAQVMNVARTSMVQAAWRRGQPLAIHAWCYGLKTGLVNDLGRTLTRIADLPEPYRLIFPDQV

SEQ ID NO: 7 - DNA, 9 bp, Artificial sequence
  DNA insert
cattcataa

SEQ ID NO: 8 - DNA, 7 bp, Artificial sequence
  DNA insert
agagaaa

SEQ ID NO: 9 - DNA, 5 bp, Artificial sequence
  DNA deletion
cgact

SEQ ID NO: 10 - DNA, 25 bp, Artificial sequence
  DNA insert
ccgccagaacgacgtggtgttggta

SEQ ID NO: 11 - DNA, 15 bp, Artificial sequence
  DNA insert
agttaaccgtggtaa

SEQ ID NO: 12 - DNA, 18 bp, Artificial sequence
  DNA insert
tcgtgtaccaatcactgc

SEQ ID NO: 13 - DNA, 6 bp, Artificial sequence
  DNA insert
ttggca

SEQ ID NO: 14 - DNA, 9 bp, Artificial sequence
  DNA insert
ttatttgat

SEQ ID NO: 15 - DNA, 12 bp, Artificial sequence
  DNA insert
attgccatatcg

SEQ ID NO: 16 - DNA, 19 bp, Artificial sequence
  DNA insert
gacgtggtgttggtagaag

SEQ ID NO: 17 - DNA, 12 bp, Artificial sequence
  DNA insert
tttacgcacgcg

SEQ ID NO: 18 - DNA, 6 bp, Artificial sequence
  DNA insert
caccta

SEQ ID NO: 19 - DNA, 9 bp, Artificial sequence
  DNA insert
attcgcgtc

SEQ ID NO: 20 - DNA, 12 bp, Artificial sequence
  DNA insert
taatgggtgaaa

SEQ ID NO: 21 - DNA, 5 bp, Artificial sequence
  DNA insert
taaga

SEQ ID NO: 22 - DNA, 5 bp, Artificial sequence
  DNA insert
ttttc

SEQ ID NO: 23 - DNA, 11 bp, Artificial sequence
  DNA insert
gatgccgagcg

SEQ ID NO: 24 - DNA, 8 bp, Artificial sequence
  DNA insert
ctttcaat

SEQ ID NO: 25 - DNA, 5 bp, Artificial sequence
  DNA deletion
ggtaa

SEQ ID NO: 26 - DNA, 9 bp, Artificial sequence
  DNA insert
tcacccatg

SEQ ID NO: 27 - DNA, 6 bp, Artificial sequence
  DNA insert
ggtgaa